European Patent Specification EP 3 819 306 B1, published January 28, 2026. Title: DENGUE VIRUS E-GLYCOPROTEIN POLYPEPTIDES CONTAINING MUTATIONS THAT ELIMINATE IMMUNODOMINANT CROSS-REACTIVE EPITOPES. Applicant: THE GOVERNMENT OF THE UNITED STATES OF AMERICA AS REPRESENTED BY THE SECRETARY OF THE DEPARTMENT OF HEALTH AND HUMAN SERVICES. Application EP12841016.4. The sequence listing filed with the application follows.

SEQUENCE LISTING (19 sequences)

SEQ ID NO: 1 - protein, 495 aa, Artificial Sequence
  Synthetic polypeptide
MRCVGIGSRDFVEGLSGATWVDVVLEHGSCVTTMAKDKPTLDIELLKTEVTNPAVLRKLCIEAKISNTTTDSRCPTQGEATLVEEQDANFVCRRTFVDRGWGNGCRDFGKGSLITCAKFKCVTKLEGKIVQYENLKYSVIVTVHTGDQHQVGNESTEHGTTATITPQAPTTEIQLTDYGALTLDCSPRTGLDFNEMVLLTMKEKSWLVHKQWFLDLPLPWTSGASTSQETWNRQDLLVTFKTAHAKKQEVVVLGSQEGAMHTALTGATEIQTSGTTTIFAGHLKCRLKMDKLTLKGMSYVMCTGSFKLEDKVAETQHGTVLVQIKYEGTDAPCKIPFSTQDEKGVTQNGRLITANPIVTDKEKQVNIEAEPPFGESYIVIGAGEKALKLSWFKKGSTLGKAFSTTLKGAQRLAALGDTAWDFGSIGGVFNSIGKAVHQVFGGAFRTLFGGMSWITQGLMGALLLWMGINARDRSIALTFLAVGGVLLFLATNVHA

SEQ ID NO: 2 - protein, 495 aa, Artificial Sequence
  Synthetic polypeptide
MRCIGMSNRDFVEGVSGGSWVDIVLEHGSCVTTMAKNKPTLDFELIKTEAKQPATLRKYCIEAKLTNTTTESRCPTQGEPSLNEEQDKRFVCKHSMVDRGWGNGCRDFGKGGIVTCAMFRCKKNMEGKVVQPENLEYTIVITPHSGEEHAVGNDTGKHGKEIKITPQSSITEAELTGYGTVTMECSPRTGLDFNEMVLLQMENKAWLVHRQWFLDLPLPWLPGADTQGSNWIQKETLVTFKNPHAKKQDVVVLGSQEGAMHTALTGATEIQMSSGNLLFTGHLKCRLRMDKLQLKGMSYSMCTGKFKVVERIAETQHGTIVIRVQYEGDGSPCKIPFEIMDLEKRHVLGRLITVNPIVTEKDSRVNIEAEPPFGDSYIIIGVEPGQLKLNWFKKGSTLGKAFSTTLKGAQRLAALGDTAWDFGSIGGVFNSIGKAVHQVFGGAFRTLFGGMSWITQGLMGALLLWMGINARDRSIALTFLAVGGVLLFLATNVHA

SEQ ID NO: 3 - protein, 493 aa, Artificial Sequence
  Synthetic polypeptide
MRCVGVGNRDFVEGLSGATWVDVVLEHGGCVTTMAKNKPTLDIELQKTEATQLATLRKLCIEGKITNITTDSRCPTQGEAILPEEQDQNYVCKHTYVDRGWGNGCDDFGKGSLVTCAKFQCLESIEGKVVQHENLKYTVIITVHTGDQHQVGNDTQGVTVEITPQASTVEAILPEYGTLGLECSPRTGLDFNEMILLTMKNKAWMVHRQWFFDLPLPWTSGATTETPTWNRKELLVTFKNAHAKKQEVVVLGSQEGAMHTALTGATEIQNSGGTSIFAGHLKCRLKMDKLELKGMSYAMCLNTFVLKDKVSETQHGTILIKVEYKGEDAPCKIPFSTEDGQGKAHNGRLITANPVVTKKEEDVNIEAEPPFGESNIVIGIGDKALKINWYKKGSTLGKAFSTTLKGAQRLAALGDTAWDFGSIGGVFNSIGKAVHQVFGGAFRTLFGGMSWITQGLMGALLLWMGINARDRSIALTFLAVGGVLLFLATNVHA

SEQ ID NO: 4 - protein, 495 aa, Artificial Sequence
  Synthetic polypeptide
MRCVGVGNRDFVEGVSGGAWVDLVLEHGGCVTTMAQGKPTLDFELIKTTAKEVALLRTYCIEASISNITTATRCPTQGEPYLKEEQDQQYICRRDVVDRGWGNGCEDFGKGGVVTCAKFSCSGKITGNLVQIENLEYTVVVTVHNGDTHAVGNDTSNHGVTATITPRSPSVEVKLPDYGELTLDCEPRSGIDFNEMILMKMKKKTWLVHKQWFLDLPLPWTAGADTSEVHWNHKERMVTFKVPHAKRQDVTVLGSQEGAMHSALTGATEVDSGDGNHMFAGHLKCKVRMEKLRIKGMSYTMCSGKFSIDDQMAETQHGTTVVKVKYEGAGAPCKVPIEIRDVNKEKVVGRIISSTPFAENTNSVTNIELEPPFGDSYIVIGVGDSALTQHWFRKGSTLGKAFSTTLKGAQRLAALGDTAWDFGSIGGVFNSIGKAVHQVFGGAFRTLFGGMSWITQGLMGALLLWMGINARDRSIALTFLAVGGVLLFLATNVHA

SEQ ID NO: 5 - protein, 685 aa, Artificial Sequence
  Synthetic polypeptide
MGKRSAGSIMWLASLAVVIAGTSAFHLTTRGGEPHMIVSKQERGKSLLFKTSAGVNMCTLIAMDLGELCEDTMTYKCPRITEAEPDDVDCWCNATDTWVTYGTCSQTGEHRRDKRSVALAPHVGLGLETRTETWMSSEGAWKQIQRVETWALRHPGFTVIALFLAHAIGTSITQKGIIFILLMLVTPSMAMRCVGIGSRDFVEGLSGATWVDVVLEHGSCVTTMAKDKPTLDIELLKTEVTNPAVLRKLCIEAKISNTTTDSRCPTQGEATLVEEQDANFVCRRTFVDRGWGNGCRDFGKGSLITCAKFKCVTKLEGKIVQYENLKYSVIVTVHTGDQHQVGNESTEHGTTATITPQAPTTEIQLTDYGALTLDCSPRTGLDFNEMVLLTMKEKSWLVHKQWFLDLPLPWTSGASTSQETWNRQDLLVTFKTAHAKKQEVVVLGSQEGAMHTALTGATEIQTSGTTTIFAGHLKCRLKMDKLTLKGMSYVMCTGSFKLEDKVAETQHGTVLVQIKYEGTDAPCKIPFSTQDEKGVTQNGRLITANPIVTDKEKQVNIEAEPPFGESYIVIGAGEKALKLSWFKKGSTLGKAFSTTLKGAQRLAALGDTAWDFGSIGGVFNSIGKAVHQVFGGAFRTLFGGMSWITQGLMGALLLWMGINARDRSIALTFLAVGGVLLFLATNVHA

SEQ ID NO: 6 - protein, 685 aa, Artificial Sequence
  Synthetic polypeptide
MGKRSAGSIMWLASLAVVIACAGAFHLTTRNGEPHMIVSRQEKGKSLLFKTEDGVNMCTLMAMDLGELCEDTITYKCPLLRQNEPEDIDCWCNSTSTWVTYGTCTTMGEHRREKRSVALVPHVGMGLETRTETWMSSEGAWKHVQRIETWILRHPGFTMMAAILAYTIGTTHFQRALIFILLTAVTPSMTMRCIGMSNRDFVEGVSGGSWVDIVLEHGSCVTTMAKNKPTLDFELIKTEAKQPATLRKYCIEAKLTNTTTESRCPTQGEPSLNEEQDKRFVCKHSMVDRGWGNGCRDFGKGGIVTCAMFRCKKNMEGKVVQPENLEYTIVITPHSGEEHAVGNDTGKHGKEIKITPQSSITEAELTGYGTVTMECSPRTGLDFNEMVLLQMENKAWLVHRQWFLDLPLPWLPGADTQGSNWIQKETLVTFKNPHAKKQDVVVLGSQEGAMHTALTGATEIQMSSGNLLFTGHLKCRLRMDKLQLKGMSYSMCTGKFKVVERIAETQHGTIVIRVQYEGDGSPCKIPFEIMDLEKRHVLGRLITVNPIVTEKDSRVNIEAEPPFGDSYIIIGVEPGQLKLNWFKKGSTLGKAFSTTLKGAQRLAALGDTAWDFGSIGGVFNSIGKAVHQVFGGAFRTLFGGMSWITQGLMGALLLWMGINARDRSIALTFLAVGGVLLFLATNVHA

SEQ ID NO: 7 - protein, 683 aa, Artificial Sequence
  Synthetic polypeptide
MGKRSAGSIMWLASLAVVIAGTSAFHLTSRDGEPRMIVGKNERGKSLLFKTASGINMCTLIAMDLGEMCDDTVTYKCPLIAEVEPEDIDCWCNLTSTWVTYGTCNQAGEHRRDKRSVALAPHVGMGLDTRTQTWMSAEGAWRQVEKVETWALRHPGFTILALFLAHYIGTSLTQKVVIFILLMLVTPSMAMRCVGVGNRDFVEGLSGATWVDVVLEHGGCVTTMAKNKPTLDIELQKTEATQLATLRKLCIEGKITNITTDSRCPTQGEAILPEEQDQNYVCKHTYVDRGWGNGCDDFGKGSLVTCAKFQCLESIEGKVVQHENLKYTVIITVHTGDQHQVGNDTQGVTVEITPQASTVEAILPEYGTLGLECSPRTGLDFNEMILLTMKNKAWMVHRQWFFDLPLPWTSGATTETPTWNRKELLVTFKNAHAKKQEVVVLGSQEGAMHTALTGATEIQNSGGTSIFAGHLKCRLKMDKLELKGMSYAMCLNTFVLKDKVSETQHGTILIKVEYKGEDAPCKIPFSTEDGQGKAHNGRLITANPVVTKKEEDVNIEAEPPFGESNIVIGIGDKALKINWYKKGSTLGKAFSTTLKGAQRLAALGDTAWDFGSIGGVFNSIGKAVHQVFGGAFRTLFGGMSWITQGLMGALLLWMGINARDRSIALTFLAVGGVLLFLATNVHA

SEQ ID NO: 8 - protein, 685 aa, Artificial Sequence
  Synthetic polypeptide
MGKRSAGSIMWLASLAVVIAGTSAFSLSTRDGEPLMIVAKHERGRPLLFKTTEGINKCTLIAMDLGEMCEDTVTYKCPLLVNTEPEDIDCWCNLTSAWVMYGTCTQSGERRREKRSVALTPHSGMGLETRAETWMSSEGAWKHAQRVESWILRNPGFALLAGFMAYMIGQTGIQRTVFFILMMLVAPSYGMRCVGVGNRDFVEGVSGGAWVDLVLEHGGCVTTMAQGKPTLDFELIKTTAKEVALLRTYCIEASISNITTATRCPTQGEPYLKEEQDQQYICRRDVVDRGWGNGCEDFGKGGVVTCAKFSCSGKITGNLVQIENLEYTVVVTVHNGDTHAVGNDTSNHGVTATITPRSPSVEVKLPDYGELTLDCEPRSGIDFNEMILMKMKKKTWLVHKQWFLDLPLPWTAGADTSEVHWNHKERMVTFKVPHAKRQDVTVLGSQEGAMHSALTGATEVDSGDGNHMFAGHLKCKVRMEKLRIKGMSYTMCSGKFSIDDQMAETQHGTTVVKVKYEGAGAPCKVPIEIRDVNKEKVVGRIISSTPFAENTNSVTNIELEPPFGDSYIVIGVGDSALTQHWFRKGSTLGKAFSTTLKGAQRLAALGDTAWDFGSIGGVFNSIGKAVHQVFGGAFRTLFGGMSWITQGLMGALLLWMGINARDRSIALTFLAVGGVLLFLATNVHA

SEQ ID NO: 9 - DNA, 5180 bp, Artificial Sequence
  Synthetic construct
gactcttcgcgatgtacgggccagatatacgcgttgacattgattattgactagttattaatagtaatcaattacggggtcattagttcatagcccatatatggagttccgcgttacataacttacggtaaatggcccgcctggctgaccgcccaacgacccccgcccattgacgtcaataatgacgtatgttcccatagtaacgccaatagggactttccattgacgtcaatgggtggagtatttacggtaaactgcccacttggcagtacatcaagtgtatcatatgccaagtacgccccctattgacgtcaatgacggtaaatggcccgcctggcattatgcccagtacatgaccttatgggactttcctacttggcagtacatctacgtattagtcatcgctattaccatggtgatgcggttttggcagtacatcaatgggcgtggatagcggtttgactcacggggatttccaagtctccaccccattgacgtcaatgggagtttgttttggcaccaaaatcaacgggactttccaaaatgtcgtaacaactccgccccattgacgcaaatgggcggtaggcgtgtacggtgggaggtctatataagcagagctctctggctaactagagaacccactgcttactggcttatcgaaattaatacgactcactatagggagacccaagctggctagcgtttaaacttaagcttggtaccgccgccgccatgggcaagaggtccgccggctcaatcatgtggctcgcgagcttggcagttgtcatagctggtacaagcgctttccatctgaccacccgagggggagagccgcacatgatagtcagcaagcaggaaagaggaaagtcacttttgtttaagacctcagcaggtgtcaacatgtgcacccttatagcgatggatttgggagagttatgtgaggacacaatgacttacaaatgccctcgaatcactgaggcggaaccagatgacgttgattgttggtgcaatgccacagacacatgggtgacctatggaacatgttcccaaactggcgagcaccgacgagacaaacgttccgtcgcactggccccacacgtgggacttggtttggaaacaagaaccgaaacgtggatgtcctctgaaggcgcttggaaacagatacaaagagtggagacttgggccctgagacacccaggattcacggtgatagccctttttctagcacatgccataggaacatccatcacccagaaagggattattttcattttgttaatgctggtaacaccatccatggccatgcgatgcgtgggaataggcagcagggacttcgtggaaggactgtcaggagcaacttgggtagatgtggtactggaacatggaagttgcgtcaccaccatggcaaaagacaaaccaacattggacattgaactcttgaagacggaagtcacaaaccctgccgtcctgcgcaaactgtgcattgaagctaaaatatcaaacaccaccaccgactcaagatgtccaacacaaggagaagccacactggtggaagaacaagacgcgaactttgtgtgtcgacgaacgtttgtggacagaggctggggcaatggctgtcgggatttcggaaaaggaagcctaataacgtgtgctaagttcaagtgtgtgacaaaactggaaggaaagatagttcaatatgaaaacttgaaatattcagtaatagtcaccgtccacactggagaccagcaccaggtgggaaatgaaagcacagaacatgggacaactgcaactataacacctcaagctcctacgacggaaatacagctgaccgactacggagctcttacattggattgttcacctagaacaggactagactttaatgaaatggtgttgttgacaatgaaagaaaaatcatggctagttcacaaacaatggtttctagacctaccactgccttggacctcgggagcttcaacatcacaagagacttggaacagacaagatttgctggtgacattcaagacagctcatgcaaagaagcaggaagtagtcgtactaggatcacaagaaggagcaatgcacactgcgttgaccggagcgacagaaatccaaacgtctggaacgacaacaatttttgcaggacacttgaaatgtagactaaagatggacaaactgactctaaaagggatgtcatatgtgatgtgcacaggctcattcaagctagaggacaaggtggctgagacccagcatggaaccgttctagtgcagattaaatacgaaggaacagatgcaccatgcaagatccctttttcgacccaagatgaaaaaggagtaacccagaatgggagattgataacagctaaccccatagtcactgacaaagaaaaacaggtcaacattgaggcagaaccgccttttggtgagagttacatcgtgataggagcaggtgaaaaagctttgaaactaagctggttcaagaaaggaagcacgctgggcaaggccttttcaacaactttgaagggagcgtaagtatcaaggttacaagacaggtttaaggagaccaatagaaactgggcttttcgtgtccttcaactgcagtgtccttcaacgaaacagagaagactcttgcgtttctgataggcacctattggtcttactgacatccactttgcctttctctccacagtcaaagactggcagcgttgggcgacacagcctgggactttggctctattggaggggtcttcaactccataggaaaagccgttcaccaagtgtttggtggtgccttcagaacactctttgggggaatgtcttggatcacacaagggctaatgggtgccctactgctctggatgggcataaacgcacgagaccgatcaattgctttgaccttcttagccgtagggggtgtgctcctgttcttagcgaccaatgtgcatgcttaattagtttgagcggccgctcgagtctagagggcccgtttaaacccgctgatcagcctcgactgtgccttctagttgccagccatctgttgtttgcccctcccccgtgccttccttgaccctggaaggtgccactcccactgtcctttcctaataaaatgaggaaattgcatcgcattgtctgagtaggtgtcattctattctggggggtggggtggggcaggacagcaagggggaggattgggaagacaatagcaggcatgctggggatgcggtgggctctatggcttctactgggcggttttatggacagcaagcgaaccggaattgccagctggggcgccctctggtaaggttgggaagccctgcaaagtaaactggatggctttctcgccgccaaggatctgatggcgcaggggatcaagctctgatcaagagacaggatgaggatcgtttcgcatgattgaacaagatggattgcacgcaggttctccggccgcttgggtggagaggctattcggctatgactgggcacaacagacaatcggctgctctgatgccgccgtgttccggctgtcagcgcaggggcgcccggttctttttgtcaagaccgacctgtccggtgccctgaatgaactgcaagacgaggcagcgcggctatcgtggctggccacgacgggcgttccttgcgcagctgtgctcgacgttgtcactgaagcgggaagggactggctgctattgggcgaagtgccggggcaggatctcctgtcatctcaccttgctcctgccgagaaagtatccatcatggctgatgcaatgcggcggctgcatacgcttgatccggctacctgcccattcgaccaccaagcgaaacatcgcatcgagcgagcacgtactcggatggaagccggtcttgtcgatcaggatgatctggacgaagagcatcaggggctcgcgccagccgaactgttcgccaggctcaaggcgagcatgcccgacggcgaggatctcgtcgtgacccatggcgatgcctgcttgccgaatatcatggtggaaaatggccgcttttctggattcatcgactgtggccggctgggtgtggcggaccgctatcaggacatagcgttggctacccgtgatattgctgaagagcttggcggcgaatgggctgaccgcttcctcgtgctttacggtatcgccgctcccgattcgcagcgcatcgccttctatcgccttcttgacgagttcttctgaattattaacgcttacaatttcctgatgcggtattttctccttacgcatctgtgcggtatttcacaccgcatacaggtggcacttttcggggaaatgtgcgcggaacccctatttgtttatttttctaaatacattcaaatatgtatccgctcatgagacaataaccctgataaatgcttcaataatagcacgtgctaaaacttcatttttaatttaaaaggatctaggtgaagatcctttttgataatctcatgaccaaaatcccttaacgtgagttttcgttccactgagcgtcagaccccgtagaaaagatcaaaggatcttcttgagatcctttttttctgcgcgtaatctgctgcttgcaaacaaaaaaaccaccgctaccagcggtggtttgtttgccggatcaagagctaccaactctttttccgaaggtaactggcttcagcagagcgcagataccaaatactgtccttctagtgtagccgtagttaggccaccacttcaagaactctgtagcaccgcctacatacctcgctctgctaatcctgttaccagtggctgctgccagtggcgataagtcgtgtcttaccgggttggactcaagacgatagttaccggataaggcgcagcggtcgggctgaacggggggttcgtgcacacagcccagcttggagcgaacgacctacaccgaactgagatacctacagcgtgagctatgagaaagcgccacgcttcccgaagggagaaaggcggacaggtatccggtaagcggcagggtcggaacaggagagcgcacgagggagcttccagggggaaacgcctggtatctttatagtcctgtcgggtttcgccacctctgacttgagcgtcgatttttgtgatgctcgtcaggggggcggagcctatggaaaaacgccagcaacgcggcctttttacggttcctgggcttttgctggccttttgctcacatgttct

SEQ ID NO: 10 - DNA, 5180 bp, Artificial Sequence
  Synthetic construct
gactcttcgcgatgtacgggccagatatacgcgttgacattgattattgactagttattaatagtaatcaattacggggtcattagttcatagcccatatatggagttccgcgttacataacttacggtaaatggcccgcctggctgaccgcccaacgacccccgcccattgacgtcaataatgacgtatgttcccatagtaacgccaatagggactttccattgacgtcaatgggtggagtatttacggtaaactgcccacttggcagtacatcaagtgtatcatatgccaagtacgccccctattgacgtcaatgacggtaaatggcccgcctggcattatgcccagtacatgaccttatgggactttcctacttggcagtacatctacgtattagtcatcgctattaccatggtgatgcggttttggcagtacatcaatgggcgtggatagcggtttgactcacggggatttccaagtctccaccccattgacgtcaatgggagtttgttttggcaccaaaatcaacgggactttccaaaatgtcgtaacaactccgccccattgacgcaaatgggcggtaggcgtgtacggtgggaggtctatataagcagagctctctggctaactagagaacccactgcttactggcttatcgaaattaatacgactcactatagggagacccaagctggctagcgtttaaacttaagcttggtaccgccgccgccatgggcaagaggtccgccggctcaatcatgtggctcgcgagcttggcagttgtcatagcttgtgcaggcgccttccatttaaccacacgtaacggagaaccacacatgatcgtcagcagacaagagaaagggaaaagtcttctgtttaaaacagaggatggcgtgaacatgtgtaccctcatggccatggaccttggtgaattgtgtgaagacacaatcacgtacaagtgtccccttctcaggcagaatgagccagaagacatagactgttggtgcaactctacgtccacgtgggtaacttatgggacgtgtaccaccatgggagaacatagaagagaaaaaagatcagtggcactcgttccacatgtgggaatgggactggagacacgaactgaaacatggatgtcatcagaaggggcctggaaacatgtccagagaattgaaacttggatcttgagacatccaggcttcaccatgatggcagcaatcctggcatacaccataggaacgacacatttccaaagagccctgattttcatcttactgacagctgtcactccttcaatgacaatgcgttgcataggaatgtcaaatagagactttgtggaaggggtttcaggaggaagctgggttgacatagtcttagaacatgggagctgtgtgacgacgatggcaaaaaacaaaccaacattggattttgaactgataaaaacagaagccaaacagcctgccaccctaaggaagtactgtatagaggcaaagctaaccaacacaacaacagaatctcgctgcccaacacaaggggaacccagcctaaatgaagagcaggacaaaaggttcgtctgcaaacactccatggtagacagaggatggggaaatggatgtcgcgactttggaaagggaggcattgtgacctgtgctatgttcagatgcaaaaagaacatggaaggaaaagttgtgcaaccagaaaacttggaatacaccattgtgataacacctcactcaggggaagagcatgcagtcggaaatgacacaggaaaacatggcaaggaaatcaaaataacaccacagagttccatcacagaagcagaattgacaggttatggcactgtcacaatggagtgctctccaagaacgggcctcgacttcaatgagatggtgttgttgcagatggaaaataaagcttggctggtgcacaggcaatggttcctagacctgccgttaccatggttgcccggagcggacacacaagggtcaaattggatacagaaagagacattggtcactttcaaaaatccccatgcgaagaaacaggatgttgttgttttaggatcccaagaaggggccatgcacacagcacttacaggggccacagaaatccaaatgtcatcaggaaacttactcttcacaggacatctcaagtgcaggctgagaatggacaagctacagctcaaaggaatgtcatactctatgtgcacaggaaagtttaaagttgtggagcgaatagcagaaacacaacatggaacaatagttatcagagtgcaatatgaaggggacggctctccatgcaagatcccttttgagataatggatttggaaaaaagacatgtcttaggtcgcctgattacagtcaacccaattgtgacagaaaaagatagccgggtcaacatagaagcagaacctccattcggagacagctacatcatcataggagtagagccgggacaactgaagctcaactggtttaagaaaggaagcacgctgggcaaggccttttcaacaactttgaagggagcgtaagtatcaaggttacaagacaggtttaaggagaccaatagaaactgggcttttcgtgtccttcaactgcagtgtccttcaacgaaacagagaagactcttgcgtttctgataggcacctattggtcttactgacatccactttgcctttctctccacagtcaaagactggcagcgttgggcgacacagcctgggactttggctctattggaggggtcttcaactccataggaaaagccgttcaccaagtgtttggtggtgccttcagaacactctttgggggaatgtcttggatcacacaagggctaatgggtgccctactgctctggatgggcataaacgcacgagaccgatcaattgctttgaccttcttagccgtagggggtgtgctcctgttcttagcgaccaatgtgcatgcttaattagtttgagcggccgctcgagtctagagggcccgtttaaacccgctgatcagcctcgactgtgccttctagttgccagccatctgttgtttgcccctcccccgtgccttccttgaccctggaaggtgccactcccactgtcctttcctaataaaatgaggaaattgcatcgcattgtctgagtaggtgtcattctattctggggggtggggtggggcaggacagcaagggggaggattgggaagacaatagcaggcatgctggggatgcggtgggctctatggcttctactgggcggttttatggacagcaagcgaaccggaattgccagctggggcgccctctggtaaggttgggaagccctgcaaagtaaactggatggctttctcgccgccaaggatctgatggcgcaggggatcaagctctgatcaagagacaggatgaggatcgtttcgcatgattgaacaagatggattgcacgcaggttctccggccgcttgggtggagaggctattcggctatgactgggcacaacagacaatcggctgctctgatgccgccgtgttccggctgtcagcgcaggggcgcccggttctttttgtcaagaccgacctgtccggtgccctgaatgaactgcaagacgaggcagcgcggctatcgtggctggccacgacgggcgttccttgcgcagctgtgctcgacgttgtcactgaagcgggaagggactggctgctattgggcgaagtgccggggcaggatctcctgtcatctcaccttgctcctgccgagaaagtatccatcatggctgatgcaatgcggcggctgcatacgcttgatccggctacctgcccattcgaccaccaagcgaaacatcgcatcgagcgagcacgtactcggatggaagccggtcttgtcgatcaggatgatctggacgaagagcatcaggggctcgcgccagccgaactgttcgccaggctcaaggcgagcatgcccgacggcgaggatctcgtcgtgacccatggcgatgcctgcttgccgaatatcatggtggaaaatggccgcttttctggattcatcgactgtggccggctgggtgtggcggaccgctatcaggacatagcgttggctacccgtgatattgctgaagagcttggcggcgaatgggctgaccgcttcctcgtgctttacggtatcgccgctcccgattcgcagcgcatcgccttctatcgccttcttgacgagttcttctgaattattaacgcttacaatttcctgatgcggtattttctccttacgcatctgtgcggtatttcacaccgcatacaggtggcacttttcggggaaatgtgcgcggaacccctatttgtttatttttctaaatacattcaaatatgtatccgctcatgagacaataaccctgataaatgcttcaataatagcacgtgctaaaacttcatttttaatttaaaaggatctaggtgaagatcctttttgataatctcatgaccaaaatcccttaacgtgagttttcgttccactgagcgtcagaccccgtagaaaagatcaaaggatcttcttgagatcctttttttctgcgcgtaatctgctgcttgcaaacaaaaaaaccaccgctaccagcggtggtttgtttgccggatcaagagctaccaactctttttccgaaggtaactggcttcagcagagcgcagataccaaatactgtccttctagtgtagccgtagttaggccaccacttcaagaactctgtagcaccgcctacatacctcgctctgctaatcctgttaccagtggctgctgccagtggcgataagtcgtgtcttaccgggttggactcaagacgatagttaccggataaggcgcagcggtcgggctgaacggggggttcgtgcacacagcccagcttggagcgaacgacctacaccgaactgagatacctacagcgtgagctatgagaaagcgccacgcttcccgaagggagaaaggcggacaggtatccggtaagcggcagggtcggaacaggagagcgcacgagggagcttccagggggaaacgcctggtatctttatagtcctgtcgggtttcgccacctctgacttgagcgtcgatttttgtgatgctcgtcaggggggcggagcctatggaaaaacgccagcaacgcggcctttttacggttcctgggcttttgctggccttttgctcacatgttct

SEQ ID NO: 11 - DNA, 3986 bp, Artificial Sequence
  Synthetic construct
gactcttcgcgatgtacgggccagatatacgcgttgacattgattattgactagttattaatagtaatcaattacggggtcattagttcatagcccatatatggagttccgcgttacataacttacggtaaatggcccgcctggctgaccgcccaacgaccccgccccattgacgtcaataatgacgtatgttcccatagtaacgccaatagggactttccattgacgtcaatgggtggagtatttacggtaaactgcccacttggcagtacatcaagtgtatcatatgccaagtacgccccctattgacgtcaatgacggtaaatggcccgcctggcattatgcccagtacatgaccttatgggactttcctacttggcagtacatctacgtattagtcatcgctattaccatggtgatgcggttttggcagtacatcaatgggcgtggatagcggtttgactcacggggatttccaagtctccaccccattgacgtcaatgggagtttgttttggcaccaaaatcaacgggactttccaaaatgtcgtaacaactccgccccattgacgcaaatgggcggtaggcgtgtacggtgggaggtctatataagcagagctctctggctaactagagaacccactgcttactggcttatcgaaattaatacgactcactatagggagacccaagctggctagcgtttaaacttaagcttggtaccgccgccgccatgggcaagaggtccgccggctcaatcatgtggctcgcgagcttggcagttgtcatagctggtacaagcgctttccacttgacttcacgagatggagagccgcgcatgatcgtggggaagaatgaaagagggaaatccctactttttaagacagcttctggaatcaacatgtgcacactcatagccatggacttgggagagatgtgtgatgacacggtcacttacaaatgccccctcattgccgaagtggaacctgaagacattgactgttggtgcaaccttacatcgacatgggtgacttatggaacgtgcaatcaagctggggagcatagacgcgacaagagatcagtggcgttagctccccatgtcggcatgggactggacacacgcacccaaacctggatgtcggctgaaggagcttggagacaagtcgagaaggtagagacatgggcccttaggcacccagggttcaccatactagctctatttcttgcccattacataggcacttccctgacccagaaagtggttatttttatactactaatgctggtcactccatccatggcaatgagatgcgtgggagtaggaaacagagattttgtggaaggtctgtcgggagctacgtgggttgatgtggtgctcgagcacggtgggtgtgtgaccaccatggctaagaacaagcctacgctggacatagagcttcagaagaccgaggccacccaactggcgaccctaaggaagttatgcattgagggaaaaattaccaacataacaactgactcaaggtgtcctacccagggggaagcgattttacctgaggagcaggaccagaactacgtatgcaagcatacatacgtggatagaggctggggaaacggttgtgacgactttggaaaaggaagcttggtgacatgcgcgaaattccaatgtttagaatcaatagagggaaaagtggtgcaacatgagaacctcaaatacactgtcatcattacagtgcacacaggagaccaacaccaggtgggaaatgacacgcagggagtcacggttgagataacaccccaggcatcaaccgttgaagctatcttgcctgaatatggaacccttgggctagaatgctcaccacggacaggtttggatttcaatgaaatgatcttattgacaatgaagaacaaagcatggatggtacatagacaatggttctttgacctacccctaccatggacatcaggagctacaacagaaacaccaacttggaacaggaaagagcttcttgtgacattcaaaaatgcacatgcaaaaaagcaagaagtagttgtccttggatcgcaagagggagcaatgcacacagcgctgacaggagctacagagatccaaaactcaggaggtacaagcatttttgcggggcacttgaaatgtagacttaagatggacaaattagaactcaaggggatgagctatgcaatgtgcttgaatacttttgtgttgaaggacaaggtctctgaaacgcagcatgggacaatactcattaaggttgagtacaaaggggaagatgcaccttgcaagattcctttctccacagaggatggacaagggaaagctcacaatggtagactgatcacagccaacccagtggtgaccaagaaggaggaggatgtcaacattgaggctgaacctccttttggggaaagtaacatagtgattggaattggagacaaagccttgaaaattaactggtacaagaagggaagcacgctgggcaaggccttttcaacaactttgaagggagcgtaagtatcaaggttacaagacaggtttaaggagaccaatagaaactgggcttttcgtgtccttcaactgcagtgtccttcaacgaaacagagaagactcttgcgtttctgataggcacctattggtcttactgacatccactttgcctttctctccacagtcaaagactggcagcgttgggcgacacagcctgggactttggctctattggaggggtcttcaactccataggaaaagccgttcaccaagtgtttggtggtgccttcagaacactctttgggggaatgtcttggatcacacaagggctaatgggtgccctactgctctggatgggcataaacgcacgagaccgatcaattgctttgaccttcttagccgtagggggtgtgctcctgttcttagcgaccaatgtgcatgcttaattagtttgagcggccgctcgagtctagagggcccgtttaaacccgctgatcagcctcgactgtgccttctagttgccagccatctgttgtttgcccctcccccgtgccttccttgaccctggaaggtgccactcccactgtcctttcctaataaaatgaggaaattgcatcgcattgtctgagtaggtgtcattctattctggggggtggggtggggcaggacagcaagggggaggattgggaagacaatagcaggcatgctggggatgcggtgggctctatggcttctactgggcggttttatggacagcaagcgaaccggaattgccagctggggcgccctctggtaaggttgggaagccctgcaaagtaaactggatggctttctcgccgccaaggatctgatggcgcaggggatcaagctctgatcaagagacaggatgaggatcgtttcgcatgattgaacaagatggattgcacgcaggttctccggccgcttgggtggagaggctattcggctatgactgggcacaacagacaatcggctgctctgatgccgccgtgttccggctgtcagcgcaggggcgcccggttctttttgtcaagaccgacctgtccggtgccctgaatgaactgcaagacgaggcagcgcggctatcgtggctggccacgacgggcgttccttgcgcagctgtgctcgacgttgtcactgaagcgggaagggactggctgctattgggcgaagtgccggggcaggatctcctgtcatctcaccttgctcctgccgagaaagtatccatcatggctgatgcaatgcggcggctgcatacgcttgatccggctacctgcccattcgaccaccaagcgaaacatcgcatcgagcgagcacgtactcggatggaagccggtcttgtcgatcaggatgatctggacgaagagcatcaggggctcgcgccagccgaactgttcgccaggctcaaggcgagcatgcccgacggcgaggatctcgtcgtgacccatggcgatgcctgcttgccgaat

SEQ ID NO: 12 - DNA, 5210 bp, Artificial Sequence
  Synthetic construct
gactcttcgcgatgtacgggccagatatacgcgttgacattgattattgactagttattaatagtaatcaattacggggtcattagttcatagcccatatatggagttccgcgttacataacttacggtaaatggcccgcctggctgaccgcccaacgacccccgcccattgacgtcaataatgacgtatgttcccatagtaacgccaatagggactttccattgacgtcaatgggtggagtatttacggtaaactgcccacttggcagtacatcaagtgtatcatatgccaagtacgccccctattgacgtcaatgacggtaaatggcccgcctggcattatgcccagtacatgaccttatgggactttcctacttggcagtacatctacgtattagtcatcgctattaccatggtgatgcggttttggcagtacatcaatgggcgtggatagcggtttgactcacggggatttccaagtctccaccccattgacgtcaatgggagtttgttttggcaccaaaatcaacgggactttccaaaatgtcgtaacaactccgccccattgacgcaaatgggcggtaggcgtgtacggtgggaggtctatataagcagagctctctggctaactagagaacccactgcttactggcttatcgaaattaatacgactcactatagggagacccaagctggctagcgtttaaacttaagcttggtaccgccgccgccatgggcaagaggtccgccggctcaatcatgtggctcgcgagcttggcagttgtcatagctggtacaagcgctttttccttgtcaacgagagatggcgaaccccttatgatagtggcgaaacacgaaagggggagacctctcttgtttaagacaacagagggaatcaacaagtgcactcttattgccatggacctgggtgaaatgtgcgaggacaccgtcacgtataaatgccctttactggtcaataccgaacccgaagacattgattgctggtgcaatctcacgtctgcctgggtcatgtatgggacatgcacccaaagtggggaacggagacgagagaagcgctcagtagctctaacaccacattcaggaatgggattggaaacaagggctgaaacatggatgtcatcggaaggagcttggaaacacgctcagagggtagagagttggatactcagaaacccaggattcgcgctcttggcaggatttatggcctatatgattgggcaaacaggaatccagcgaacagtcttctttattttaatgatgctggtcgccccatcctacggaatgcgatgcgtaggagtggggaacagagacttcgtggaaggagtctcaggtggagcatgggtcgatctggtgctagaacatggaggatgtgtcacaactatggcccagggaaaaccaaccttggattttgaactgatcaagacaacagccaaggaagtggctctattaagaacctattgcattgaagcctctatatcaaacataaccacggcaacaagatgtccaacgcaaggagagccttacctcaaagaggaacaagatcaacagtacatctgccggagagacgtggtagacagagggtggggcaatggctgtgaagactttgggaaaggaggagttgtgacatgtgcgaagttttcatgctcggggaagataacaggcaacttagtccaaattgagaaccttgaatacacagtggttgtaacagtccacaatggagacacccatgcagtaggaaatgacacatccaaccacggagtgacagccacgataacccccaggtcaccatcggtagaagttaaattgccggactatggagaattgacactcgattgtgaacccaggtccggaattgactttaatgagatgattctgatgaaaatgaaaaagaaaacgtggcttgtgcacaagcaatggtttttggatctacctctaccatggacagcaggagcagacacgtcagaagttcattggaatcacaaagagagaatggtgacgttcaaggtccctcatgctaagagacaggatgtgacagtgctaggatctcaggaaggagccatgcattcagccctcaccggagccacagaagtggattccggtgatggaaaccacatgtttgccggacatttgaagtgcaaagttcgcatggagaaattgaggatcaagggaatgtcgtacacgatgtgctcaggaaagttctcaattgatgaccagatggcagaaacacagcatgggacaacagtggtaaaagtcaagtatgagggtgctggagctccatgtaaagttcccatagagataagagatgtgaacaaggaaaaagtggttgggcgtatcatctcatctaccccttttgctgagaataccaacagtgtgaccaatatagaattggaacccccttttggggatagctacatagtgataggtgtgggagacagtgcactaacacagcattggttcaggaaagggagtacgctgggcaaggccttttcaacaactttgaagggagcgtaagtatcaaggttacaagacaggtttaaggagaccaatagaaactgggcttttcgtgtccttcaactgcagtgtccttcaacgaaacagagaagactcttgcgtttctgataggcacctattggtcttactgacatccactttgcctttctctccacagtcaaagactggcagcgttgggcgacacagcctgggactttggctctattggaggggtcttcaactccataggaaaagccgttcaccaagtgtttggtggtgccttcagaacactctttgggggaatgtcttggatcacacaagggctaatgggtgccctactgctctggatgggcataaacgcacgagaccgatcaattgctttgaccttcttagccgtagggggtgtgctcctgttcttagcgaccaatgtgcatgcttaattagtttgagcggccgctcgagcatgcatctagagggccctattctatagtgtcacctaaatgctagagctcgctgatcagcctcgactgtgccttctagttgccagccatctgttgtttgcccctcccccgtgccttccttgaccctggaaggtgccactcccactgtcctttcctaataaaatgaggaaattgcatcgcattgtctgagtaggtgtcattctattctggggggtgggggtggggcaggacagcaagggggaggattgggaagacaatagcaggcatgctggggatgcggtgggctctatggcttctactgggcggttttatggacagcaagcgaaccggaattgccagctggggcgccctctggtaaggttgggaagccctgcaaagtaaactggatggctttctcgccgccaaggatctgatggcgcaggggatcaagctctgatcaagagacaggatgaggatcgtttcgcatgattgaacaagatggattgcacgcaggttctccggccgcttgggtggagaggctattcggctatgactgggcacaacagacaatcggctgctctgatgccgccgtgttccggctgtcagcgcaggggcgcccggttctttttgtcaagaccgacctgtccggtgccctgaatgaactgcaagacgaggcagcgcggctatcgtggctggccacgacgggcgttccttgcgcagctgtgctcgacgttgtcactgaagcgggaagggactggctgctattgggcgaagtgccggggcaggatctcctgtcatctcaccttgctcctgccgagaaagtatccatcatggctgatgcaatgcggcggctgcatacgcttgatccggctacctgcccattcgaccaccaagcgaaacatcgcatcgagcgagcacgtactcggatggaagccggtcttgtcgatcaggatgatctggacgaagagcatcaggggctcgcgccagccgaactgttcgccaggctcaaggcgagcatgcccgacggcgaggatctcgtcgtgacccatggcgatgcctgcttgccgaatatcatggtggaaaatggccgcttttctggattcatcgactgtggccggctgggtgtggcggaccgctatcaggacatagcgttggctacccgtgatattgctgaagagcttggcggcgaatgggctgaccgcttcctcgtgctttacggtatcgccgctcccgattcgcagcgcatcgccttctatcgccttcttgacgagttcttctgaattattaacgcttacaatttcctgatgcggtattttctccttacgcatctgtgcggtatttcacaccgcatacaggtggcacttttcggggaaatgtgcgcggaacccctatttgtttatttttctaaatacattcaaatatgtatccgctcatgagacaataaccctgataaatgcttcaataatagcacgtgctaaaacttcatttttaatttaaaaggatctaggtgaagatcctttttgataatctcatgaccaaaatcccttaacgtgagttttcgttccactgagcgtcagaccccgtagaaaagatcaaaggatcttcttgagatcctttttttctgcgcgtaatctgctgcttgcaaacaaaaaaaccaccgctaccagcggtggtttgtttgccggatcaagagctaccaactctttttccgaaggtaactggcttcagcagagcgcagataccaaatactgtccttctagtgtagccgtagttaggccaccacttcaagaactctgtagcaccgcctacatacctcgctctgctaatcctgttaccagtggctgctgccagtggcgataagtcgtgtcttaccgggttggactcaagacgatagttaccggataaggcgcagcggtcgggctgaacggggggttcgtgcacacagcccagcttggagcgaacgacctacaccgaactgagatacctacagcgtgagctatgagaaagcgccacgcttcccgaagggagaaaggcggacaggtatccggtaagcggcagggtcggaacaggagagcgcacgagggagcttccagggggaaacgcctggtatctttatagtcctgtcgggtttcgccacctctgacttgagcgtcgatttttgtgatgctcgtcaggggggcggagcctatggaaaaacgccagcaacgcggcctttttacggttcctgggcttttgctggccttttgctcacatgttctt

SEQ ID NO: 13 - DNA, 36 bp, Artificial Sequence
  Synthetic polynucleotide
ttcctttccgaagagacgacagccattgccccagcc

SEQ ID NO: 14 - DNA, 35 bp, Artificial Sequence
  Synthetic polynucleotide
ttccttttccgaaatccccacagccattgccccag

SEQ ID NO: 15 - DNA, 38 bp, Artificial Sequence
  Synthetic polynucleotide
cttccttttccgaaatcccgacagccattgccccagcc

SEQ ID NO: 16 - DNA, 35 bp, Artificial Sequence
  Synthetic polynucleotide
agccacttcgtcctctagcttgaatgagcctgtgc

SEQ ID NO: 17 - DNA, 37 bp, Artificial Sequence
  Synthetic polynucleotide
tcagccacctttttctctagcttgaatgagcctgtgc

SEQ ID NO: 18 - DNA, 42 bp, Artificial Sequence
  Synthetic polynucleotide
gggtctcagccaccttgtcctctagcttgaatgagcctgtgc

SEQ ID NO: 19 - DNA, 41 bp, Artificial Sequence
  Synthetic polynucleotide
gcctcaatgttgacctgtttttctttgtcagtgactatggg